European Patent Application EP 4 464 724 A1, published November 20, 2024. Title: CHIMERIC PROTEIN PRODUCTION PROCESS, CHIMERIC PROTEIN, GENE, IMMUNOGENIC COMPOSITION AND USES. Applicant: Universidade Federal de Minas Gerais. Application BR BR1020220007330, filed January 14, 2022. The sequence listing filed with the application follows.

SEQUENCE LISTING (2 sequences)

SEQ ID NO: 1 - protein, 623 aa, synthetic construct
MSDNGPQNQRNAPRITFGGPSDSTGSNQNGERSGARSKQRRPQGLPNNTASWFTALTQHGKEDLKFPRGQGVPINTNSSPDDQIGYYRRATRRIRGGDGKMKDLSPRWYFYYLGTGPEAGLPYGANKDGIIWVATEGALNTPKDHIGTRNPANNAAIVLQLPQGTTLPKGFYAEGSRGGSQASSRSSSRSRNSSRNSTPGSSRGTSPARMAGNGGDAALALLLLDRLNQLESKMSGKGQQQQGQTVTKKSAAEASKKPRQKRTATKAYNVTQAFGRRGPEQTQGNFGDQELIRQGTDYKHWPQIAQFAPSASAFFGMSRIGMEVTPSGTWLTYTGAIKLDDKDPNFKDQVILLNKHIDAYKTFPPTEPKKDKKKKADETQALPQRQKKQQTVTLLPAADLDDFSKQLQQSMSSADSTQAGGGGGMTNLCPFGEVFNATRFASVYAWNRKRISNCVADYSVLYNSASFSTFKCYGVSPTKLNDLCFTNVYADSFVIRGDEVRQIAPGQTGKIADYNYKLPDDFTGCVIAWNSNNLDSKVGGNYNYLYRLFRKSNLKPFERDISTEIYQAGSTPCNGVEGFNCYFPLQSYGFQPTNGVGYQPYRVVVLSFELLHAPATVCGPKKS

SEQ ID NO: 2 - DNA, 1872 bp, synthetic construct
  source 1..1872: mol_type = other DNA
atgagcgacaatggtccgcagaatcagcgtaatgcgccgcgtatcacctttggtggtccgagcgacagcaccggcagcaatcagaatggtgaacgtagcggtgcgcgtagcaagcaacgtcgtccgcaaggtctgccgaacaacaccgcgagctggttcaccgcgctgacccaacacggcaaggaagacctgaagtttccgcgtggtcagggcgttccgatcaacaccaacagcagcccggacgatcagattggctactatcgtcgtgcgacccgtcgtatccgtggtggcgatggtaaaatgaaggatctgagcccgcgttggtatttctattacctgggtaccggcccggaagcgggtctgccgtatggtgcgaacaaggacggcattatctgggtggcgaccgaaggtgcgctgaacaccccgaaggaccacattggtacccgtaacccggcgaacaacgcggcgatcgttctgcaactgccgcaaggtaccaccctgccgaaaggcttctacgcggagggtagccgtggtggcagccaagcgagcagccgtagcagcagccgtagccgtaacagcagccgtaacagcaccccgggtagcagccgtggtaccagcccggcgcgtatggcgggcaacggtggtgatgcggcgctggcgctgctgctgctggatcgtctgaaccaactggaaagcaagatgagcggcaaaggtcaacagcaacaaggccagaccgttaccaagaaaagcgcggcggaagcgagcaagaaaccgcgtcagaagcgtaccgcgaccaaggcgtacaacgttacccaggcgtttggtcgtcgtggtccggaacaaacccagggtaacttcggtgatcaagagctgatccgtcagggtaccgactacaaacactggccgcagatcgcgcaatttgcgccgagcgcgagcgcgttctttggtatgagccgtatcggtatggaagtgaccccgagcggtacctggctgacctacaccggtgcgatcaagctggatgacaaagacccgaacttcaaggaccaagtgatcctgctgaacaagcacatcgatgcgtacaaaaccttcccgccgaccgaaccgaagaaagacaaaaagaagaaagcggacgagacccaggcgctgccgcaacgtcagaaaaagcagcaaaccgttaccctgctgccggcggcggatctggatgacttcagcaagcagctgcaacagagcatgagcagcgcggatagcacccaagcgggtggcggcggtggcatgaccaacctgtgcccgttcggcgaagttttcaacgcgacccgtttcgcgagcgtttatgcgtggaaccgtaagcgtatcagcaactgcgttgcggactacagcgttctgtacaacagcgcgagcttcagcaccttcaaatgctacggtgttagcccgaccaaactgaacgacctgtgctttaccaacgtgtacgcggatagcttcgtgatccgtggtgatgaagtgcgtcagatcgcgccgggtcaaaccggcaaaatcgcggactataactacaagctgccggacgatttcaccggctgcgttattgcgtggaacagcaacaacctggatagcaaagtgggtggtaactataactacctgtaccgtctgttccgtaagagcaacctgaagccgttcgagcgtgatatcagcaccgagatctaccaggcgggtagcaccccgtgcaacggtgttgagggtttcaactgctacttcccgctgcagagctacggcttccaaccgaccaacggtgttggttaccagccgtatcgtgttgttgtgctgagctttgaactgctgcatgcgccggcgaccgtgtgcggcccgaagaagagctaa